European Patent Application EP 4 428 235 A1, published September 11, 2024. Title: SPINACH PLANT COMPRISING A NOVEL LOCUS FOR DOWNY MILDEW RESISTANCE. Applicant: Sakata Seed Corporation. Application JP. The sequence listing filed with the application follows.

SEQUENCE LISTING (77 sequences)

SEQ ID NO: 1 - DNA, 22 bp, synthetic construct
  source 1..22: mol_type = other DNA
gggttatctcaaatcactgccc

SEQ ID NO: 2 - DNA, 19 bp, synthetic construct
  source 1..19: mol_type = other DNA
tgaaggttggctgcgttca

SEQ ID NO: 3 - DNA, 119 bp, Spinacia tetrandra
  source 1..119: mol_type = genomic DNA
gaaaattgaatactcttatacaatgacaagtctgcccatggggatgcagtacttaacctctctccaaaccctcgaactaaaatgttgtgatgaattgaattcccttccagaatggataa

SEQ ID NO: 4 - DNA, 122 bp, Spinacia tetrandra
  source 1..122: mol_type = genomic DNA
gaacctcacctcccttcagacacttgacatatggcagtgtccagacctagctgaaagatgcagaaaacccaaaggcaaggactatcccaaaattcaacacatccccggaattgtaagtgatt

SEQ ID NO: 5 - DNA, 325 bp, Spinacia tetrandra
  source 1..325: mol_type = genomic DNA
gagattcctgagggttttttttcgttggggttggttttcatgtatatgttgctgattaaataccagactgatgatgatgatgtgtttatgggttttaaatcagattaaatatatgggaaatgtaagttaattggggatgcacataaggtgtttgatgaaatgtctattagaaatgttgtttcttggacttagaatgatatacactgtcgtcctttggtttccaatctggaatttggtttttgttttcttagtttgtttctttattccacactagcccattttttttaaactacctgcaactactaaatttcatttaccctgtatc

SEQ ID NO: 6 - DNA, 119 bp, Spinacia sp.
  source 1..119: mol_type = genomic DNA
gagaattaaagactctgacaaaatgacaagtttgcccatggggatgcagtacttaacctccctccaaaccctctatctacaccattgttatgaattgaattcccttccagaatggataa

SEQ ID NO: 7 - DNA, 122 bp, Spinacia sp.
  source 1..122: mol_type = genomic DNA
gaacctcacctcccttcagacacttgggatatcggattgtccagacctagttaaaagatgcagaaaacccaacggcaaggactatcccaaaattcaacacatccccaaaattgtaagtcatt

SEQ ID NO: 8 - DNA, 214 bp, Spinacia sp.
  source 1..214: mol_type = genomic DNA
gagattcctggggttttctttttgttggggttggatttcatgtatatgttgctgattaaatacgagactgatgatgatgatgtgtttatgggttttaaatcagattaaatatatgggaaatgtaagttagttggggatgcacataaggtgtttgatgaaatgtctatgagaaatgttgtttcttggacttagaatgatatacactgtcgtcctt

SEQ ID NO: 9 - DNA, 119 bp, Spinacia sp.
  source 1..119: mol_type = genomic DNA
ggaaattaattactctgacaaaatgacaagttttcccatggggatgcagtacttaacctccctccaaaccatccatctttatgattgttataaattgaattccattccagaatggataa

SEQ ID NO: 10 - DNA, 104 bp, Spinacia sp.
  source 1..104: mol_type = genomic DNA
gaacctcacctcccttcagagacttacgatatggcagtgtccagacctaattgaaagatgcaaagaacctaacggggaggactatcccaaaattgtaagtcatt

SEQ ID NO: 11 - DNA, 305 bp, Spinacia sp.
  source 1..305: mol_type = genomic DNA
ttcgttggggttggttttcatgtatatgttgctgattaaataccagactgatgatgatgatgtgtttatgggttttaaatcagattaaatatatgggaaatgtaagttaattggggatgcacataaggtgtttgatgaaatgtctattagaaatgttgtttcttggacttagaatgatatacactgtcgtcctttggtttccaatctggaatttggtttttgttttcttagtttgtttctttattccacactagcccattttttttaaactacctgcaactactgaatttcatttaccctgtatc

SEQ ID NO: 12 - DNA, 119 bp, Spinacia sp.; identical to SEQ ID NO: 9
  source 1..119: mol_type = genomic DNA

SEQ ID NO: 13 - DNA, 104 bp, Spinacia sp.; identical to SEQ ID NO: 10
  source 1..104: mol_type = genomic DNA

SEQ ID NO: 14 - DNA, 256 bp, Spinacia sp.
  source 1..256: mol_type = genomic DNA
gagattcctggggttttctttttgttggggttggatttcatgtatatgttgctgattaaatacgagactgatgatgatgatgatgtgtttatgggttttaaatcagattaaatatatgggaaatgtaagttaatttgggatgcacataaggtgtttgctgaaatgtctatgagaaatgttgtttcttggacttagaatgatatacactgtcgtccattggtttccaatcttacatttggtttgtgttttcttagtt

SEQ ID NO: 15 - DNA, 119 bp, Spinacia sp.
  source 1..119: mol_type = genomic DNA
gaaaattgaatactcttataaaatgacaagtctgcccatggggatgcagtacttaacctccctccaaaccctcgaactaaaatgttgtgatgaattgaattcccttccagaatggataa

SEQ ID NO: 16 - DNA, 122 bp, Spinacia sp.
  source 1..122: mol_type = genomic DNA
gaacctcacctcccttcagagacttgtgataagagaatgtcgagacctagctgaaagatgcgaagaacccaatggggaagactatcacaaaattcaacacatccccaaaattgtaagtgatt

SEQ ID NO: 17 - DNA, 45 bp, Spinacia sp.
  source 1..45: mol_type = genomic DNA
ttttttaaactacctgcaactactaattttcatttaccctgtatc

SEQ ID NO: 18 - DNA, 119 bp, Spinacia sp.; identical to SEQ ID NO: 15
  source 1..119: mol_type = genomic DNA

SEQ ID NO: 19 - DNA, 122 bp, Spinacia sp.; identical to SEQ ID NO: 16
  source 1..122: mol_type = genomic DNA

SEQ ID NO: 20 - DNA, 45 bp, Spinacia sp.; identical to SEQ ID NO: 17
  source 1..45: mol_type = genomic DNA

SEQ ID NO: 21 - DNA, 119 bp, Spinacia sp.; identical to SEQ ID NO: 15
  source 1..119: mol_type = genomic DNA

SEQ ID NO: 22 - DNA, 110 bp, Spinacia sp.
  source 1..110: mol_type = genomic DNA
gaacctcacctcccttcagagacttgtgataagagaatgtcgagacctagctgaaagatgcgaagaacccaatggggaagactatcacaaaattcaacacatccccaaaa

SEQ ID NO: 23 - DNA, 22 bp, Spinacia sp.
  source 1..22: mol_type = genomic DNA
tttcttagatttaccctgtatc

SEQ ID NO: 24 - DNA, 119 bp, Spinacia sp.; identical to SEQ ID NO: 6
  source 1..119: mol_type = genomic DNA

SEQ ID NO: 25 - DNA, 122 bp, Spinacia sp.; identical to SEQ ID NO: 7
  source 1..122: mol_type = genomic DNA

SEQ ID NO: 26 - DNA, 269 bp, Spinacia sp.
  source 1..269: mol_type = genomic DNA
gagattcgtggggttttctttttgttggggttggatttcatgtatatgttgctgattgaatacgagactgatgatgatgatgtgtttaatttatgggttttaaatcagattaaatatatgggaaatgtaagttaattggggatgcacataaggtgtttgatgaaatgtctattagaaatgttgtttcttggacttagaatgatatacactgtcgtcctttggtttccaatctggaatttgcaactactaaatttcatttaccctgtatc

SEQ ID NO: 27 - DNA, 119 bp, Spinacia sp.
  source 1..119: mol_type = genomic DNA
gagaattgaagactctgacaaaatgacaagtttgcccatggggatgcagtacttaacctccctccaaaccctctatctatcatattgtgatgaattgaattcccttccagaatggataa

SEQ ID NO: 28 - DNA, 122 bp, Spinacia sp.
  source 1..122: mol_type = genomic DNA
gaacctcacctcccttcagagacttgagatacatcattgtccagacctagctgaaagatgcagaaaacccaacggggaggactatcccaaaattcaacacatccccggcattgtaagtgatt

SEQ ID NO: 29 - DNA, 325 bp, Spinacia sp.
  source 1..325: mol_type = genomic DNA
gagattcctggggtttttttttcgttggggttggttttcatgtatatgttgctgattaaataccagactgatgatgatgatgtgtttatgggttttaaatcagattaaatatatgggaaatgtaagttagttggggatgcacataaggtgtttgatgaaatgtctattagaaatgttgtttcttggacttagaatgatatacactgtcgtcctttggtttccaatcttacatttggtttgtgttttcttagtttgtttctttaatcaacaccagcccattttttttaaactacctgcaactactaattttcatttaccctgtatc

SEQ ID NO: 30 - DNA, 119 bp, Spinacia sp.; identical to SEQ ID NO: 27
  source 1..119: mol_type = genomic DNA

SEQ ID NO: 31 - DNA, 122 bp, Spinacia sp.; identical to SEQ ID NO: 28
  source 1..122: mol_type = genomic DNA

SEQ ID NO: 32 - DNA, 325 bp, Spinachia sp.; identical to SEQ ID NO: 29
  source 1..325: mol_type = genomic DNA

SEQ ID NO: 33 - DNA, 119 bp, Spinacia sp.
  source 1..119: mol_type = genomic DNA
ggaaattgaaaactcttacaaaatgacaagtttgcccatggggatgcagtacttaacctccctccaaaccctctatctacaccattgttatgaattgaattcccttccagaatggataa

SEQ ID NO: 34 - DNA, 122 bp, Spinacia sp.; identical to SEQ ID NO: 7
  source 1..122: mol_type = genomic DNA

SEQ ID NO: 35 - DNA, 266 bp, Spinacia sp.
  source 1..266: mol_type = genomic DNA
gagattcctggggttttctttttgttggggttggatttcatgtatatgttgctgattaaatacgagactgatgatgatgatgtgtttatgggttttaaatcagattaaatatatgggaaatgtaagttagttggggatgcacataaggtgtttgatggtttccaatctggaatttggtttttgttttcttagtttgtttctttattccacactagcccattttttttaaactacctgcaactactgaatttcatttaccctgtatc

SEQ ID NO: 36 - DNA, 119 bp, Spinacia sp.
  source 1..119: mol_type = genomic DNA
ggaaattaaaggctcttgcaaaatgacaagtttgcccatggggatgcagtacttaacctccctccaaaccctccatctatcatattgtgatgaattgaattcccttccagaatggataa

SEQ ID NO: 37 - DNA, 122 bp, Spinacia sp.
  source 1..122: mol_type = genomic DNA
gaacctcacctcccttcagagacttgagatacagcattgtccagacctagctgaaagatgcagaaaacccaacggggaggactatcccaaaattcaacacatccccaaaattgtaagtcatt

SEQ ID NO: 38 - DNA, 243 bp, Spinacia sp.
  source 1..243: mol_type = genomic DNA
attggggttggttttcatgtatatgttgctgattaaataccagactgatgatgatgatgtgtttatgggttttaaatcagattaaatatatgggaaatgtaagttaattggggatgcacataaggtgtttgatgaaatgtctatgagaaatgttgtttcttggacttagaatgatatacactgtcgtcctttggtttccaatcttacatttggtttgtgttttcttagtttgtttcttgtatc

SEQ ID NO: 39 - DNA, 119 bp, Spinacia sp.; identical to SEQ ID NO: 6
  source 1..119: mol_type = genomic DNA

SEQ ID NO: 40 - DNA, 122 bp, Spinacia sp.
  source 1..122: mol_type = genomic DNA
gaacctcacctcccttcagagacttacgatatggcagtgtccagacctaattgaaagatgcaaagaacctaacggggaggactatcccaaaattcaacacatccccaaaattgtaagtcatt

SEQ ID NO: 41 - DNA, 328 bp, Spinacia sp.
  source 1..328: mol_type = genomic DNA
gagattcctggggttttctttttgttggggttggatttcatgtatatgttgctgattaaatacgagactgatgatgatgatgatgtgtttatgggttttaaatcagattaaatatatgggaaatgtaagttaatttgggatgcacataaggtgtttgctgaaatgtctatgagaaatgttgtttcttggacttagaatgatatacactgtcgtccattggtttccaatcttacatttggtttgtgttttcttagtttgtttctttaatcaacaccaacccatttttttaaaactacctgcaactactaatttacgttgaccctgtatc

SEQ ID NO: 42 - DNA, 119 bp, Spinacia sp.
  source 1..119: mol_type = genomic DNA
gagaattgaagactctgacaaaatgacaagttttcccatggggatgcagtacttaacctccctccaaaccatccatctttatgattgttataaattgaattccattccagaatggataa

SEQ ID NO: 43 - DNA, 122 bp, Spinacia sp.; identical to SEQ ID NO: 40
  source 1..122: mol_type = genomic DNA

SEQ ID NO: 44 - DNA, 180 bp, Spinacia sp.
  source 1..180: mol_type = genomic DNA
gagatagactgatgatgatgatgtgtttaatttatgggttttaaatcagattaaatatatgggaaatgtaagttaattggggatgcacataaggtgtttgatgaaatgtctattagaaatgttgtttcttggacttagaatgatatacactgtcgtcctttggtttccaatcttacattt

SEQ ID NO: 45 - DNA, 119 bp, Spinacia sp.
  source 1..119: mol_type = genomic DNA
gagaattgaagactctgacaaaatgacaagtttgcccatggggatgcagtacttaacctccctccaaaccctctatctacaccattgttatgaattgaattcccttccagaatggataa

SEQ ID NO: 46 - DNA, 122 bp, Spinacia sp.; identical to SEQ ID NO: 40
  source 1..122: mol_type = genomic DNA

SEQ ID NO: 47 - DNA, 265 bp, Spinacia sp.
  source 1..265: mol_type = genomic DNA
gagatcctggatgatgatgatgtgtttatgggttttaaatcagattaaatatatgggaaatgtaagttaattggggatgcacataaggtgtttgatgaaatgtctatgagaaatgttgtttcttggacttagaatgatatacactgtcgtcctttggtttccaatcttacatttggtttgtgttttcttagtttgtttctttaatcaacaccagcccattttttttaaactacctgcaactactaattttcatttaccctgtatc

SEQ ID NO: 48 - DNA, 119 bp, Spinacia sp.; identical to SEQ ID NO: 6
  source 1..119: mol_type = genomic DNA

SEQ ID NO: 49 - DNA, 122 bp, Spinacia sp.; identical to SEQ ID NO: 40
  source 1..122: mol_type = genomic DNA

SEQ ID NO: 50 - DNA, 268 bp, Spinacia sp.
  source 1..268: mol_type = genomic DNA
gaggagactgatgatgatgatgatgtgtttatgggttttaaatcagattaaatatatgggaaatgtaagttaatttgggatgcacataaggtgtttgctgaaatgtctatgagaaatgttgtttcttggacttagaatgatatacactgtcgtccattggtttccaatcttacatttggtttgtgttttcttagtttgtttctttaatcaacaccaacccatttttttaaaactacctgcaactactaatttacgttgaccctgtatc

SEQ ID NO: 51 - DNA, 119 bp, Spinacia sp.; identical to SEQ ID NO: 6
  source 1..119: mol_type = genomic DNA

SEQ ID NO: 52 - DNA, 122 bp, Spinacia sp.
  source 1..122: mol_type = genomic DNA
gaacctcacctcccttcagagacttacgatatggcagtgtccagacctaattgaaagatgcgaagaacccaacggcgaggactatcccaaaattcaacacatccccaaaattgtaagtcatt

SEQ ID NO: 53 - DNA, 331 bp, Spinacia sp.
  source 1..331: mol_type = genomic DNA
gagattcctggggttttctttttgttggggttggatttcatgtatatgttgctgattaaatacgagactgatgatgatgatgatgatgtgtttatgggttttaaatcagattaaatatatgggaaatgtaagttaatttgggatgcacataaggtgtttgctgaaatgtctatgagaaatgttgtttcttggacttagaatgatatacactgtcgtccattggtttccaatcttacatttggtttgtgttttcttagtttgtttctttaatcaacaccaacccatttttttaaaactacctgcaactactaatttacgttgaccctgtatc

SEQ ID NO: 54 - DNA, 119 bp, Spinacia sp.; identical to SEQ ID NO: 6
  source 1..119: mol_type = genomic DNA

SEQ ID NO: 55 - DNA, 122 bp, Spinacia sp.
  source 1..122: mol_type = genomic DNA
gaacctcacctcccttcagacacttgggatatcggattgtccagacctagttaaaagatgcagaaaacccaacggcaaggactatcccaaaattcaacacatcccctattggagtatagaac

SEQ ID NO: 56 - DNA, 265 bp, Spinacia sp.
  source 1..265: mol_type = genomic DNA
gagattcctggggttttctttttgttggggttggatttcatgtatatgttgctgattaaatacgagactgatgatgatgatgtgtttatgggttttaaatcagattaaatatatgggaaatgcaagttaatttgggatgcacataaggtgtttgctgaaatgtctatgagaaatgttgtttcttggacttagaatgatatacactgtcgtcctttggtttccaatcttacatcctgcaactactaatttacgtttaccctgtatc

SEQ ID NO: 57 - DNA, 119 bp, Spinacia sp.
  source 1..119: mol_type = genomic DNA
gagaattaaagactctgacaaaatgacaagtttgcccatggggatgcagtacttaacctccctccaaaccctcgaactatcatattgtgatgaattgaattcccttccagaatggataa

SEQ ID NO: 58 - DNA, 122 bp, Spinacia sp.
  source 1..122: mol_type = genomic DNA
gaacctcacctcccttcagacacttgggatatcggattgtccagacctagttaaaatatgcagaaaacccaacggcgaggactatcccaaaattcaacacatccccggcattgtaagtgatt

SEQ ID NO: 59 - DNA, 266 bp, Spinacia sp.
  source 1..266: mol_type = genomic DNA
atacgagactgatgatgattatgtgtttatgggttttaaatcagattaaatatatggaaaatgtaagttagttggggatgcacataaggtgtttgatgaaatgtcttttagaaatgttgtttcttggacttagaatgatatacactgtcgtcctttggtttccaatcttacatttggtttgtgttttcttagtttgtttctttaatcaacaccaacccattttttttaaactacctgcaactactaatttacgtttaccctttatc

SEQ ID NO: 60 - DNA, 119 bp, Spinacia sp.
  source 1..119: mol_type = genomic DNA
ggaaattaaatactctgacaaaatgacaagtttgcccatggggatgcagtacttaacctccctccaaaccatccatctttattgttgtggtaaattgaattccattccagaatggataa

SEQ ID NO: 61 - DNA, 65 bp, Spinacia sp.
  source 1..65: mol_type = genomic DNA
gaacctcacctcccttcagagcgactatcccaaaattcaacacatccccaaaattgtaagtcatt

SEQ ID NO: 62 - DNA, 325 bp, Spinacia sp.
  source 1..325: mol_type = genomic DNA
gagattcctggggttttctttttgttggggttggttttcatgtatatgttgctgattaaatacgagactgatgatgattatgtgtttatgggttttaaatcagattaaatatatggaaaatgtaagttagttggggatgcacataaggtgtttgatgaaatgtctattagaaatgttgtttcttggacttagaatgatatacactgtcgtcctttggtttccaatcttacatttggtttgtgttttcttagtttgtttctttaatcaacaccagcccattttttttaaactacctgcaactactaattttcatttaccctgtatc

SEQ ID NO: 63 - DNA, 119 bp, Spinacia sp.
  source 1..119: mol_type = genomic DNA
ggaaattaaaggctcttgcaaaatgacaagtttgcccatggggatgcagtacttaacctccctccaaaccctcgaactatcatattgtgatgaattgaattcccttccagaatggataa

SEQ ID NO: 64 - DNA, 122 bp, Spinacia sp.; identical to SEQ ID NO: 58
  source 1..122: mol_type = genomic DNA

SEQ ID NO: 65 - DNA, 325 bp, Spinacia sp.
  source 1..325: mol_type = genomic DNA
gagattcctggggtttttttttcgttggggttggttttcatgtatatgttgctgattaaatacgagactgatgatgattatgtgtttatgggttttaaatcagattaaatatatggaaaatgtaagttagttggggatgcacataaggtgtttgatgaaatgtctattagaaatgttgtttcttggacttagaatgatatacactgtcgtcctttggtttccaatcttacatttggtttgtgttttcttagtttgtttctttaatcaacaccaacccattttttttaaactacctgcaactactaatttacgtttaccctttatc

SEQ ID NO: 66 - DNA, 119 bp, Spinacia sp.
  source 1..119: mol_type = genomic DNA
ggaaattaaaggctcttgcaaaatgacaagtttgcccatggggatgcagtacttaacctccctccaaaccctcaaactagaaaattgtgatgaattgaattcccttccagaatggataa

SEQ ID NO: 67 - DNA, 122 bp, Spinacia sp.
  source 1..122: mol_type = genomic DNA
gaacctcacctcccttcagagacttgtgatacggctgtgtccagacctagttaaaagatgcggaaaacccaaaggcaaggactatcccaaaattcaacacatccccgaaattgtaagtgatt

SEQ ID NO: 68 - DNA, 286 bp, Spinacia sp.
  source 1..286: mol_type = genomic DNA
tatatgttgctgattaaatacgagactgatgatgatgatgatgtgtttatgggttttaaatcagattaaatatatgggaaatgtaagttaatttgggatgcacataaggtgtttgctgaaatgtctatgagaaatgttgtttcttggacttagaatgatatacactgtcgtccattggtttccaatcttacatttggtttgtgttttcttagtttgtttctttaatcaacaccaacccatttttttaaaactacctgcaactactaatttacgttgaccctgtatc

SEQ ID NO: 69 - DNA, 119 bp, Spinacia sp.; identical to SEQ ID NO: 57
  source 1..119: mol_type = genomic DNA

SEQ ID NO: 70 - DNA, 122 bp, Spinacia sp.; identical to SEQ ID NO: 7
  source 1..122: mol_type = genomic DNA

SEQ ID NO: 71 - DNA, 325 bp, Spinacia sp.
  source 1..325: mol_type = genomic DNA
gagattcctggggttttctttttgttggggttggatttcatgtatatgttgctgattaaatacgagactgatgatgatgatgtgtttatgggttttaaatcagattaaatatatgggaaatgcaagttaatttgggatgcacataaggtgtttgctgaaatgtctatgagaaatgttgtttcttggacttagaatgatatacactgtcgtcctttggtttccaatcttacatttggtttgtgttttcttagtttgtttctttaatcaacaccaacccgttttttttaaactacctgcaactactaatttacgtttaccctgtatc

SEQ ID NO: 72 - DNA, 119 bp, Spinacia sp.; identical to SEQ ID NO: 57
  source 1..119: mol_type = genomic DNA

SEQ ID NO: 73 - DNA, 122 bp, Spinacia sp.; identical to SEQ ID NO: 7
  source 1..122: mol_type = genomic DNA

SEQ ID NO: 74 - DNA, 242 bp, Spinacia sp.
  source 1..242: mol_type = genomic DNA
atggggttggatttcatgtatatgttgctgattaaatacgagactgatgatgatgatgtgtttatgggttttaaatcagattaaatatatgggaaatgcaagttaatttgggatgcacataaggtgtttgctgaaatgtctatgagaaatgttgtttcttggacttagaatgatatacactgtcgtcctttggtttccaatcttacatttggtttgtgttttcttagtttgtttcttgtatc

SEQ ID NO: 75 - DNA, 119 bp, Spinacia sp.; identical to SEQ ID NO: 6
  source 1..119: mol_type = genomic DNA

SEQ ID NO: 76 - DNA, 122 bp, Spinacia sp.
  source 1..122: mol_type = genomic DNA
gaacctcacctcccttcagagccttgtgatacggcggtgtccagacctaattgaaagatgcgaagaacccaacggcgaggactatcccaaaattcgacacatctccagaattgtaagtcatt

SEQ ID NO: 77 - DNA, 326 bp, Spinacia sp.
  source 1..326: mol_type = genomic DNA
gagattcctggggttttttttttcgttggggttggttttcatgtatatgttgctgattaaatacgagactgatgatgatgatgtgtttatgggttttaaatcagattaaatatatgggaaatgcaagttaatttgggatgcacataaggtgtttgctgaaatgtctatgagaaatgttgtttcttggacttagaatgatatacactgtcgtcctttggtttccaatcttacatttggtttgtgttttcttagtttgtttctttaatcaacaccaacccgttttttttaaactacctgcaactactaatttacgtttaccctgtatc